European Patent Specification EP 4 340 868 B1, published July 9, 2025. Title: Secreted splicing variant of Klotho for treating bone disorders. Applicant: Universitat Autonoma de Barcelona Institució Catalana de Recerca i Estudis Avançats Universitat de Barcelona Fundació Hospital Universitari Vall D'hebron - Institut De Recerca. The sequence listing filed with the application follows.

SEQUENCE LISTING (15 sequences)

SEQ ID NO: 1 - protein, 549 aa, Homo sapiens
MPASAPPRRPRPPPPSLSLLLVLLGLGGRRLRAEPGDGAQTWARVSRPPAPEAAGLFQGTFPDGFLWAVGSAAYQTEGGWQQHGKGASIWDTFTHHPLAPPGDSRNASLPLGAPSPLQPATGDVASDSYNNVFRDTEALRELGVTHYRFSISWARVLPNGSAGVPNREGLRYYRRLLERLRELGVQPVVTLYHWDLPQRLQDAYGGWANRALADHFRDYAELCFRHFGGQVKYWITIDNPYVVAWHGYATGRLAPGIRGSPRLGYLVAHNLLLAHAKVWHLYNTSFRPTQGGQVSIALSSHWINPRRMTDHSIKECQKSLDFVLGWFAKPVFIDGDYPESMKNNLSSILPDFTESEKKFIKGTADFFALCFGPTLSFQLLDPHMKFRQLESPNLRQLLSWIDLEFNHPQIFIVENGWFVSGTTKRDDAKYMYYLKKFIMETLKAIKLDGVDVIGYTAWSLMDGFEWHRGYSIRRGLFYVDFLSQDKMLLPKSSALFYQKLIEKNGFPPLPENQPLEGTFPCDFAWGVVDNYIQVSQLTKPISSLTKPYH

SEQ ID NO: 2 - protein, 550 aa, Mus musculus
MLARAPPRRPPRLVLLRLLLLHLLLLALRARCLSAEPGQGAQTWARFARAPAPEAAGLLHDTFPDGFLWAVGSAAYQTEGGWRQHGKGASIWDTFTHHSGAAPSDSPIVVAPSGAPSPPLSSTGDVASDSYNNVYRDTEGLRELGVTHYRFSISWARVLPNGTAGTPNREGLRYYRRLLERLRELGVQPVVTLYHWDLPQRLQDTYGGWANRALADHFRDYAELCFRHFGGQVKYWITIDNPYVVAWHGYATGRLAPGVRGSSRLGYLVAHNLLLAHAKVWHLYNTSFRPTQGGRVSIALSSHWINPRRMTDYNIRECQKSLDFVLGWFAKPIFIDGDYPESMKNNLSSLLPDFTESEKRLIRGTADFFALSFGPTLSFQLLDPNMKFRQLESPNLRQLLSWIDLEYNHPPIFIVENGWFVSGTTKRDDAKYMYYLKKFIMETLKAIRLDGVDVIGYTAWSLMDGFEWHRGYSIRRGLFYVDFLSQDKELLPKSSALFYQKLIEDNGFPPLPENQPLEGTFPCDFAWGVVDNYVQLSPLTKPSVGLLLPH

SEQ ID NO: 3 - DNA, 1650 bp, Homo sapiens
atgcccgccagcgccccgccgcgccgcccgcgtccaccgccgccgtcgctgtcgctgctgctggtgctgctgggcctgggcggacgacgcctgcgtgcggagccgggcgacggcgcgcagacctgggcccgtgtctcgcggcctcctgcccccgaggccgcgggcctcttccagggcaccttccccgacggcttcctctgggccgtgggcagcgccgcctaccagaccgagggcggctggcagcagcacggcaagggtgcgtccatctgggacacgttcacccaccaccccctggcacccccgggagactcccggaacgccagtctgccgttgggcgccccgtcgccgctgcagcccgccaccggggacgtagccagcgacagctacaacaacgtcttccgcgacacggaggcgctgcgcgagctcggggtcactcactaccgcttctccatctcgtgggcgcgagtgctccccaatggcagcgcgggcgtccccaaccgcgaggggctgcgctactaccggcgcctgctggagcggctgcgggagctgggcgtgcagcccgtggtcaccctgtaccactgggacctgccccagcgcctgcaggacgcctacggcggctgggccaaccgcgccctggccgaccacttcagggattacgcggagctctgcttccgccacttcggcggtcaggtcaagtactggatcaccatcgacaacccctacgtggtggcctggcacggctacgccaccgggcgcctggcccccggcatccggggcagcccgcggctcgggtacctggtggcgcacaacctcctcctggctcatgccaaagtctggcatctctacaatacttctttccgtcccactcagggaggtcaggtgtccattgccctaagctctcactggatcaatcctcgaagaatgaccgaccacagcatcaaagaatgtcaaaaatctctggactttgtactaggttggtttgccaaacccgtatttattgatggtgactatcccgagagcatgaagaataacctttcatctattctgcctgattttactgaatctgagaaaaagttcatcaaaggaactgctgacttttttgctctttgctttggacccaccttgagttttcaacttttggaccctcacatgaagttccgccaattggaatctcccaacctgaggcaactgctttcctggattgaccttgaatttaaccatcctcaaatatttattgtggaaaatggctggtttgtctcagggaccaccaagagagatgatgccaaatatatgtattacctcaaaaagttcatcatggaaaccttaaaagccatcaagctggatggggtggatgtcatcgggtataccgcatggtccctcatggatggtttcgagtggcacagaggttacagcatcaggcgtggactcttctatgttgactttctaagccaggacaagatgttgttgccaaagtcttcagccttgttctaccaaaagctgatagagaaaaatggcttccctcctttacctgaaaatcagcccctagaagggacatttccctgtgactttgcttggggagttgtcgacaactacattcaagtaagtcagctgacaaaaccaatcagcagtctcaccaagccctatcactag

SEQ ID NO: 4 - DNA, 1653 bp, Mus musculus
atgctcgcccgcgcccctcctcgccgcccgccgcggctggtgctgctccgtttgctgttgctgcatctgctgctgctcgccctgcgcgcccgctgcctgagcgctgagccgggtcagggcgcgcagacctgggctcgcttcgcgcgcgctcctgccccagaggccgctggcctcctccacgacaccttccccgacggtttcctctgggcggtaggcagcgccgcctatcagaccgagggcggctggcgacagcacggcaaaggcgcgtccatctgggacactttcacccatcactctggggcggccccgtccgactccccgatcgtcgtggcgccgtcgggtgccccgtcgcctcccctgtcctccactggagatgtggccagcgatagttacaacaacgtctaccgcgacacagaggggctgcgcgaactgggggtcacccactaccgcttctccatatcgtgggcgcgggtgctccccaatggcaccgcgggcactcccaaccgcgaggggctgcgctactaccggcggctgctggagcggctgcgggagctgggcgtgcagccggtggttaccctgtaccattgggacctgccacagcgcctgcaggacacctatggcggatgggccaatcgcgccctggccgaccatttcagggattatgccgagctctgcttccgccacttcggtggtcaggtcaagtactggatcaccattgacaacccctacgtggtggcctggcacgggtatgccaccgggcgcctggccccgggcgtgaggggcagctccaggctcgggtacctggttgcccacaacctacttttggctcatgccaaagtctggcatctctacaacacctctttccgccccacacagggaggccgggtgtctatcgccttaagctcccattggatcaatcctcgaagaatgactgactataatatcagagaatgccagaagtctcttgactttgtgctaggctggtttgccaaacccatatttattgatggcgactacccagagagtatgaagaacaacctctcgtctcttctgcctgattttactgaatctgagaagaggctcatcagaggaactgctgacttttttgctctctccttcggaccaaccttgagctttcagctattggaccctaacatgaagttccgccaattggagtctcccaacctgaggcagcttctgtcttggatagatctggaatataaccaccctccaatatttattgtggaaaatggctggtttgtctcgggaaccaccaaaagggatgatgccaaatatatgtattatctcaagaagttcataatggaaaccttaaaagcaatcagactggatggggtcgacgtcattgggtacaccgcgtggtcgctcatggacggtttcgagtggcataggggctacagcatccggcgaggactcttctacgttgactttctgagtcaggacaaggagctgttgccaaagtcttcggccttgttctaccaaaagctgatagaggacaatggctttcctcctttacctgaaaaccagccccttgaagggacatttccctgtgactttgcttggggagttgttgacaactacgttcagctgagtcctttgacaaaacccagtgtcggcctcttgcttcctcactaa

SEQ ID NO: 5 - protein, 534 aa, Homo sapiens
MPASAPPRRPRPPPPSLSLLLVLLGLGGRRLRAEPGDGAQTWARVSRPPAPEAAGLFQGTFPDGFLWAVGSAAYQTEGGWQQHGKGASIWDTFTHHPLAPPGDSRNASLPLGAPSPLQPATGDVASDSYNNVFRDTEALRELGVTHYRFSISWARVLPNGSAGVPNREGLRYYRRLLERLRELGVQPVVTLYHWDLPQRLQDAYGGWANRALADHFRDYAELCFRHFGGQVKYWITIDNPYVVAWHGYATGRLAPGIRGSPRLGYLVAHNLLLAHAKVWHLYNTSFRPTQGGQVSIALSSHWINPRRMTDHSIKECQKSLDFVLGWFAKPVFIDGDYPESMKNNLSSILPDFTESEKKFIKGTADFFALCFGPTLSFQLLDPHMKFRQLESPNLRQLLSWIDLEFNHPQIFIVENGWFVSGTTKRDDAKYMYYLKKFIMETLKAIKLDGVDVIGYTAWSLMDGFEWHRGYSIRRGLFYVDFLSQDKMLLPKSSALFYQKLIEKNGFPPLPENQPLEGTFPCDFAWGVVDNYIQV

SEQ ID NO: 6 - protein, 536 aa, Mus musculus
MLARAPPRRPPRLVLLRLLLLHLLLLALRARCLSAEPGQGAQTWARFARAPAPEAAGLLHDTFPDGFLWAVGSAAYQTEGGWRQHGKGASIWDTFTHHSGAAPSDSPIVVAPSGAPSPPLSSTGDVASDSYNNVYRDTEGLRELGVTHYRFSISWARVLPNGTAGTPNREGLRYYRRLLERLRELGVQPVVTLYHWDLPQRLQDTYGGWANRALADHFRDYAELCFRHFGGQVKYWITIDNPYVVAWHGYATGRLAPGVRGSSRLGYLVAHNLLLAHAKVWHLYNTSFRPTQGGRVSIALSSHWINPRRMTDYNIRECQKSLDFVLGWFAKPIFIDGDYPESMKNNLSSLLPDFTESEKRLIRGTADFFALSFGPTLSFQLLDPNMKFRQLESPNLRQLLSWIDLEYNHPPIFIVENGWFVSGTTKRDDAKYMYYLKKFIMETLKAIRLDGVDVIGYTAWSLMDGFEWHRGYSIRRGLFYVDFLSQDKELLPKSSALFYQKLIEDNGFPPLPENQPLEGTFPCDFAWGVVDNYVQV

SEQ ID NO: 7 - DNA, 3683 bp, Artificial
  Gene construct
ggcattgattattgactagttattaatagtaatcaattacggggtcattagttcatagcccatatatggagttccgcgttacataacttacggtaaatggcccgcctggctgaccgcccaacgacccccgcccattgacgtcaataatgacgtatgttcccatagtaacgccaatagggactttccattgacgtcaatgggtggagtatttacggtaaactgcccacttggcagtacatcaagtgtatcatatgccaagtacgccccctattgacgtcaatgacggtaaatggcccgcctggcattatgcccagtacatgaccttatgggactttcctacttggcagtacatctacgtattagtcatcgctattaccatggtcgaggtgagccccacgttctgcttcactctccccatctcccccccctccccacccccaattttgtatttatttattttttaattattttgtgcagcgatgggggcggggggggggggggggcgcgcgccaggcggggcggggcggggcgaggggcggggcggggcgaggcggagaggtgcggcggcagccaatcagagcggcgcgctccgaaagtttccttttatggcgaggcggcggcggcggcggccctataaaaagcgaagcgcgcggcgggcgggagtcgctgcgttgccttcgccccgtgccccgctccgcgccgcctcgcgccgcccgccccggctctgactgaccgcgttactcccacaggtgagcgggcgggacggcccttctcctccgggctgtaattagcgcttggtttaatgacggcttgtttcttttctgtggctgcgtgaaagccttgaggggctccgggagggccctttgtgcggggggagcggctcggggggtgcgtgcgtgtgtgtgtgcgtggggagcgccgcgtgcggctccgcgctgcccggcggctgtgagcgctgcgggcgcggcgcggggctttgtgcgctccgcagtgtgcgcgaggggagcgcggccgggggcggtgccccgcggtgcggggggctgcgaggggaacaaaggctgcgtgcggggtgtgtgcgtgggggggtgagcagggggtgtgggcgcgtcggtcgggctgcaaccccccctgcacccccctccccgagttgctgagcacggcccggcttcgggtgcggggctccgtacggggcgtggcgcggggctcgccgtgccgggcggggggtggcggcaggtgggggtgccgggcggggcggggccgcctcgggccggggagggctcgggggaggggcgcggcggcccccggagcgccggcggctgtcgaggcgcggcgagccgcagccattgccttttatggtaatcgtgcgagagggcgcagggacttcctttgtcccaaatctgtgcggagccgaaatctgggaggcgccgccgcaccccctctagcgggcgcggggcgaagcggtgcggcgccggcaggaaggaaatgggcggggagggccttcgtgcgtcgccgcgccgccgtccccttctccctctccagcctcggggctgtccgcggggggacggctgccttcgggggggacggggcagggcggggttcggcttctggcgtgtgaccggcggctctagagcctctgctaaccatgttcatgccttcttctttttcctacagctcctgggcaacgtgctggttattgtgctgtctcatcattttggcaaagaattgattaattcgagcgaacgcgtcgagtcgctcggtacgatttaaattgaattggcctcgagcgcaagcttgagctagcctcgacctcgagacgcgtgatatcggatccactagtccagtgtggtggaattcgccgccaccatgctagcccgcgcccctcctcgccgcccgccgcggctggtgctgctccgtttgctgttgctgcatctgctgctgctcgccctgcgcgcccgctgcctgagcgctgagccgggtcagggcgcgcagacctgggctcgcttcgcgcgcgctcctgccccagaggccgctggcctcctccacgacaccttccccgacggtttcctctgggcggtaggcagcgccgcctatcagaccgagggcggctggcgacagcacggcaaaggcgcgtccatctgggacactttcacccatcactctggggcggccccgtccgactccccgatcgtcgtggcgccgtcgggtgccccgtcgcctcccctgtcctccactggagatgtggccagcgatagttacaacaacgtctaccgcgacacagaggggctgcgcgaactgggggtcacccactaccgcttctccatatcgtgggcgcgggtgctccccaatggcaccgcgggcactcccaaccgcgaggggctgcgctactaccggcggctgctggagcggctgcgggagctgggcgtgcagccggtggttaccctgtaccattgggacctgccacagcgcctgcaggacacctatggcggatgggccaatcgcgccctggccgaccatttcagggattatgccgagctctgcttccgccacttcggtggtcaggtcaagtactggatcaccattgacaacccctacgtggtggcctggcacgggtatgccaccgggcgcctggccccgggcgtgaggggcagctccaggctcgggtacctggttgcccacaacctacttttggctcatgccaaagtctggcatctctacaacacctctttccgccccacacagggaggccgggtgtctatcgccttaagctcccattggatcaatcctcgaagaatgactgactataatatcagagaatgccagaagtctcttgactttgtgctaggctggtttgccaaacccatatttattgatggcgactacccagagagtatgaagaacaacctctcgtctcttctgcctgattttactgaatctgagaagaggctcatcagaggaactgctgacttttttgctctctccttcggaccaaccttgagctttcagctattggaccctaacatgaagttccgccaattggagtctcccaacctgaggcagcttctgtcttggatagatctggaatataaccaccctccaatatttattgtggaaaatggctggtttgtctcgggaaccaccaaaagggatgatgccaaatatatgtattatctcaagaagttcataatggaaaccttaaaagcaatcagactggatggggtcgacgtcattgggtacaccgcgtggtcgctcatggacggtttcgagtggcataggggctacagcatccggcgaggactcttctacgttgactttctgagtcaggacaaggagctgttgccaaagtcttcggccttgttctaccaaaagctgatagaggacaatggctttcctcctttacctgaaaaccagccccttgaagggacatttccctgtgactttgcttggggagttgttgacaactacgttcagctgagtcctttgacaaaacccagtgtcggcctcttgcttcctcactaagggccgcttccctttagtgagggttaatgcttcgagcagacatgataagatacattgatgagtttggacaaaccacaactagaatgcagtgaaaaaaatgctttatttgtgaaatttgtgatgctattgctttatttgtaaccattataagctgcaataaacaagtt

SEQ ID NO: 8 - DNA, 2494 bp, Artificial
  Gene construct
ggcattgattattgactagttattaatagtaatcaattacggggtcattagttcatagcccatatatggagttccgcgttacataacttacggtaaatggcccgcctggctgaccgcccaacgacccccgcccattgacgtcaataatgacgtatgttcccatagtaacgccaatagggactttccattgacgtcaatgggtggagtatttacggtaaactgcccacttggcagtacatcaagtgtatcatatgccaagtccgccccctattgacgtcaatgacggtaaatggcccgcctggcattatgcccagtacatgaccttacgggactttcctacttggcagtacatctacgtattagtcatcgctattaccatggtgatgcggttttggcagtacaccaatgggcgtggatagcggtttgactcacggggatttccaagtctccaccccattgacgtcaatgggagtttgttttggcaccaaaatcaacgggactttccaaaatgtcgtaacaactgcgatcgcccgccccgttgacgcaaatgggcggtaggcgtgtacggtgggaggtctatataagcagagctctctggctaactagagaacccactgcttactggcttatcgaaattaatacgactcactatagggagacccaagctggctagaatgctcgcccgcgcccctcctcgccgcccgccgcggctggtgctgctccgtttgctgttgctgcatctgctgctgctcgccctgcgcgcccgctgcctgagcgctgagccgggtcagggcgcgcagacctgggctcgcttcgcgcgcgctcctgccccagaggccgctggcctcctccacgacaccttccccgacggtttcctctgggcggtaggcagcgccgcctatcagaccgagggcggctggcgacagcacggcaaaggcgcgtccatctgggacactttcacccatcactctggggcggccccgtccgactccccgatcgtcgtggcgccgtcgggtgccccgtcgcctcccctgtcctccactggagatgtggccagcgatagttacaacaacgtctaccgcgacacagaggggctgcgcgaactgggggtcacccactaccgcttctccatatcgtgggcgcgggtgctccccaatggcaccgcgggcactcccaaccgcgaggggctgcgctactaccggcggctgctggagcggctgcgggagctgggcgtgcagccggtggttaccctgtaccattgggacctgccacagcgcctgcaggacacctatggcggatgggccaatcgcgccctggccgaccatttcagggattatgccgagctctgcttccgccacttcggtggtcaggtcaagtactggatcaccattgacaacccctacgtggtggcctggcacgggtatgccaccgggcgcctggccccgggcgtgaggggcagctccaggctcgggtacctggttgcccacaacctacttttggctcatgccaaagtctggcatctctacaacacctctttccgccccacacagggaggccgggtgtctatcgccttaagctcccattggatcaatcctcgaagaatgactgactataatatcagagaatgccagaagtctcttgactttgtgctaggctggtttgccaaacccatatttattgatggcgactacccagagagtatgaagaacaacctctcgtctcttctgcctgattttactgaatctgagaagaggctcatcagaggaactgctgacttttttgctctctccttcggaccaaccttgagctttcagctattggaccctaacatgaagttccgccaattggagtctcccaacctgaggcagcttctgtcttggatagatctggaatataaccaccctccaatatttattgtggaaaatggctggtttgtctcgggaaccaccaaaagggatgatgccaaatatatgtattatctcaagaagttcataatggaaaccttaaaagcaatcagactggatggggtcgacgtcattgggtacaccgcgtggtcgctcatggacggtttcgagtggcataggggctacagcatccggcgaggactcttctacgttgactttctgagtcaggacaaggagctgttgccaaagtcttcggccttgttctaccaaaagctgatagaggacaatggctttcctcctttacctgaaaaccagccccttgaagggacatttccctgtgactttgcttggggagttgttgacaactacgttcagctgagtcctttgacaaaacccagtgtcggcctcttgcttcctcactaagggccgcttccctttagtgagggttaatgcttcgagcagacatgataagatacattgatgagtttggacaaaccacaactagaatgcagtgaaaaaaatgctttatttgtgaaatttgtgatgctattgctttatttgtaaccattataagctgcaataaacaagtt

SEQ ID NO: 9 - DNA, 4071 bp, Artificial
  Gene construct
ggcattgattattgactagttattaatagtaatcaattacggggtcattagttcatagcccatatatggagttccgcgttacataacttacggtaaatggcccgcctggctgaccgcccaacgacccccgcccattgacgtcaataatgacgtatgttcccatagtaacgccaatagggactttccattgacgtcaatgggtggagtatttacggtaaactgcccacttggcagtacatcaagtgtatcatatgccaagtccgccccctattgacgtcaatgacggtaaatggcccgcctggcattatgcccagtacatgaccttacgggactttcctacttggcagtacatctacgtattagtcatcgctattaccatggtgatgcggttttggcagtacaccaatgggcgtggatagcggtttgactcacggggatttccaagtctccaccccattgacgtcaatgggagtttgttttggcaccaaaatcaacgggactttccaaaatgtcgtaacaactgcgatcgcccgccccgttgacgcaaatgggcggtaggcgtgtacggtgggaggtctatataagcagagctcgtttagtgaaccgtcagatcactagaagcttgatatcgaattcgcccttgataatcattgctcgtggggcggcgggagcgggggtgggcaccgcgtagggagggcggcggggcgcgggcatataggggcgcggcgcggtgccctcccggctcccgcagcatgctagcccgcgcccctcctcgccgcccgccgcggctggtgctgctccgtttgctgttgctgcatctgctgctgctcgccctgcgcgcccgctgcctgagcgctgagccgggtcagggcgcgcagacctgggctcgcttcgcgcgcgctcctgccccagaggccgctggcctcctccacgacaccttccccgacggtttcctctgggcggtaggcagcgccgcctatcagaccgagggcggctggcgacagcacggcaaaggcgcgtccatctgggacactttcacccatcactctggggcggccccgtccgactccccgatcgtcgtggcgccgtcgggtgccccgtcgcctcccctgtcctccactggagatgtggccagcgatagttacaacaacgtctaccgcgacacagaggggctgcgcgaactgggggtcacccactaccgcttctccatatcgtgggcgcgggtgctccccaatggcaccgcgggcactcccaaccgcgaggggctgcgctactaccggcggctgctggagcggctgcgggagctgggcgtgcagccggtggttaccctgtaccattgggacctgccacagcgcctgcaggacacctatggcggatgggccaatcgcgccctggccgaccatttcagggattatgccgagctctgcttccgccacttcggtggtcaggtcaagtactggatcaccattgacaacccctacgtggtggcctggcacgggtatgccaccgggcgcctggccccgggcgtgaggggcagctccaggctcgggtacctggttgcccacaacctacttttggctcatgccaaagtctggcatctctacaacacctctttccgccccacacagggaggccgggtgtctatcgccttaagctcccattggatcaatcctcgaagaatgactgactataatatcagagaatgccagaagtctcttgactttgtgctaggctggtttgccaaacccatatttattgatggcgactacccagagagtatgaagaacaacctctcgtctcttctgcctgattttactgaatctgagaagaggctcatcagaggaactgctgacttttttgctctctccttcggaccaaccttgagctttcagctattggaccctaacatgaagttccgccaattggagtctcccaacctgaggcagcttctgtcttggatagatctggaatataaccaccctccaatatttattgtggaaaatggctggtttgtctcgggaaccaccaaaagggatgatgccaaatatatgtattatctcaagaagttcataatggaaaccttaaaagcaatcagactggatggggtcgacgtcattgggtacaccgcgtggtcgctcatggacggtttcgagtggcataggggctacagcatccggcgaggactcttctacgttgactttctgagtcaggacaaggagctgttgccaaagtcttcggccttgttctaccaaaagctgatagaggacaatggctttcctcctttacctgaaaaccagccccttgaagggacatttccctgtgactttgcttggggagttgttgacaactacgttcaagtggacactactctctctcagtttactgacccgaatgtctatctgtgggatgtgcatcacagtaagaggcttattaaagtagacggggttgtagccaagaagagaaaaccttactgtgttgatttctctgccatccggcctcagataaccttacttcgagaaatgcgggtcacccactttcgcttctccctggactgggccctgatcttgcctctgggtaaccagacccaagtgaaccacacggttctgcacttctaccgctgcatgatcagcgagctggtgcacgccaacatcactccagtggtggccctgtggcagccagcagccccgcaccaaggcctgccacatgcccttgcaaaacatggggcctgggagaacccgcacactgctctggcgtttgcagactacgcaaacctgtgttttaaagagttgggtcactgggtcaatctctggatcaccatgaacgagccaaacacacggaacatgacctatcgtgccgggcaccacctcctgagagcccatgccttggcttggcatctgtacgatgacaagtttagggcggctcagaaaggcaaaatatccatcgccttgcaggctgactggatagaaccggcctgccctttctctcaaaatgacaaagaagtggccgagagagttttggaatttgatataggctggctggcagagcctatttttggttccggagattatccacgtgtgatgagggactggctgaaccaaaaaaacaattttcttttgccctatttcaccgaagatgaaaaaaagctagtccggggttcctttgacttcctggcggtgagtcattacaccaccattctggtagactgggaaaaggaggatccgatgaaatacaacgattacttggaggtacaggagatgactgacatcacatggctcaactctcccagtcaggtggcagtggtgccttgggggctgcgcaaagtgctcaactggctaaggttcaagtacggagacctcccgatgtatgtgacagccaatggaatcgatgatgacccccacgccgagcaagactcactgaggatctattatattaagaattatgtgaatgaggctctgaaagcctacgtgttggacgacatcaacctttgtggctactttgcgtattcacttagtgatcgctcagctcccaagtctggcttttatcgatatgctgcgaatcagtttgagcccaaaccatctatgaaacattacaggaaaattattgacagcaatggcttcctgggttctggaacactgggaaggttttgtccagaagaatacactgtgtgcaccgaatgtggattttttcaaacccggaagtctttgctggtcttcatctcgtttcttgtttttacttttattatttctcttgctctcatttttcactactccaagaaaggccagagaagttataagtaatgtgaacgtctgcctggccattcgctttgggatcaagatgtacacgccgtcagccgtttgcacctctctgtgttgtgagccgcattccacacatttcgattctagagcggccgcttccctttagtgagggttaatgcttcgagcagacatgataagatacattgatgagtttggacaaaccacaactagaatgcagtgaaaaaaatgctttatttgtgaaatttgtgatgctattgctttatttgtaaccattataagctgcaataaacaagtt

SEQ ID NO: 10 - DNA, 1157 bp, Artificial
  Gene construct
ggcattgattattgactagttattaatagtaatcaattacggggtcattagttcatagcccatatatggagttccgcgttacataacttacggtaaatggcccgcctggctgaccgcccaacgacccccgcccattgacgtcaataatgacgtatgttcccatagtaacgccaatagggactttccattgacgtcaatgggtggagtatttacggtaaactgcccacttggcagtacatcaagtgtatcatatgccaagtccgccccctattgacgtcaatgacggtaaatggcccgcctggcattatgcccagtacatgaccttacgggactttcctacttggcagtacatctacgtattagtcatcgctattaccatggtgatgcggttttggcagtacaccaatgggcgtggatagcggtttgactcacggggatttccaagtctccaccccattgacgtcaatgggagtttgttttggcaccaaaatcaacgggactttccaaaatgtcgtaacaactgcgatcgcccgccccgttgacgcaaatgggcggtaggcgtgtacggtgggaggtctatataagcagagctcgtttagtgaaccgtcagatcactagaagctttattgcggtagtttatcacagttaaattgctaacgcagtcagtgcttctgacacaacagtctcgaacttaagctgcagtgactctcttaaggtagccttgcagaagttggtcgtgaggcactgggcaggtaagtatcaaggttacaagacaggtttaaggagaccaatagaaactgggcttgtcgagacagagaagactcttgcgtttctgataggcacctattggtcttactgacatccactttgcctttctctccacaggtgtccactcccagttcaattacagctcttaaggctagagtacttaatacgactcactataggctagcctcgacctcgagacgcgtgatatcggatccgtcgacgcggccgcttccctttagtgagggttaatgcttcgagcagacatgataagatacattgatgagtttggacaaaccacaactagaatgcagtgaaaaaaatgctttatttgtgaaatttgtgatgctattgctttatttgtaaccattataagctgcaataaacaagtt

SEQ ID NO: 11 - protein, 1014 aa, Mus musculus
MLARAPPRRPPRLVLLRLLLLHLLLLALRARCLSAEPGQGAQTWARFARAPAPEAAGLLHDTFPDGFLWAVGSAAYQTEGGWRQHGKGASIWDTFTHHSGAAPSDSPIVVAPSGAPSPPLSSTGDVASDSYNNVYRDTEGLRELGVTHYRFSISWARVLPNGTAGTPNREGLRYYRRLLERLRELGVQPVVTLYHWDLPQRLQDTYGGWANRALADHFRDYAELCFRHFGGQVKYWITIDNPYVVAWHGYATGRLAPGVRGSSRLGYLVAHNLLLAHAKVWHLYNTSFRPTQGGRVSIALSSHWINPRRMTDYNIRECQKSLDFVLGWFAKPIFIDGDYPESMKNNLSSLLPDFTESEKRLIRGTADFFALSFGPTLSFQLLDPNMKFRQLESPNLRQLLSWIDLEYNHPPIFIVENGWFVSGTTKRDDAKYMYYLKKFIMETLKAIRLDGVDVIGYTAWSLMDGFEWHRGYSIRRGLFYVDFLSQDKELLPKSSALFYQKLIEDNGFPPLPENQPLEGTFPCDFAWGVVDNYVQVDTTLSQFTDPNVYLWDVHHSKRLIKVDGVVAKKRKPYCVDFSAIRPQITLLREMRVTHFRFSLDWALILPLGNQTQVNHTVLHFYRCMISELVHANITPVVALWQPAAPHQGLPHALAKHGAWENPHTALAFADYANLCFKELGHWVNLWITMNEPNTRNMTYRAGHHLLRAHALAWHLYDDKFRAAQKGKISIALQADWIEPACPFSQNDKEVAERVLEFDIGWLAEPIFGSGDYPRVMRDWLNQKNNFLLPYFTEDEKKLVRGSFDFLAVSHYTTILVDWEKEDPMKYNDYLEVQEMTDITWLNSPSQVAVVPWGLRKVLNWLRFKYGDLPMYVTANGIDDDPHAEQDSLRIYYIKNYVNEALKAYVLDDINLCGYFAYSLSDRSAPKSGFYRYAANQFEPKPSMKHYRKIIDSNGFLGSGTLGRFCPEEYTVCTECGFFQTRKSLLVFISFLVFTFIISLALIFHYSKKGQRSYK

SEQ ID NO: 12 - DNA, 20 bp, Artificial
  oligo
ctgccccattgacaaaaggc

SEQ ID NO: 13 - DNA, 19 bp, Artificial
  oligo
ctcaccgtcggtcatcagc

SEQ ID NO: 14 - DNA, 20 bp, Artificial
  oligo
gcacagtttacgttgccgac

SEQ ID NO: 15 - DNA, 19 bp, Artificial
  oligo
cgttagcaatccgcaagca